European Patent Application EP 4 470 555 A1, published December 4, 2024. Title: Anti-tag chimeric antigen receptors with specificity for mutated peptides derived from human FGFR2. Applicant: Miltenyi Biotec B.V. & Co. KG. Application EP. The sequence listing filed with the application follows.

SEQUENCE LISTING (5 sequences)

SEQ ID NO: 1 - protein, 10 aa, synthetic construct
DVVERSPHRP

SEQ ID NO: 2 - protein, 10 aa, synthetic construct
DVVERWPHRP

SEQ ID NO: 3 - protein, 10 aa, synthetic construct
YVVERWRHRP

SEQ ID NO: 4 - protein, 248 aa, synthetic construct
QVQLVQSGAEVKKPGSSVKVSCKASGGTFSSYAISWVRQAPGQGLEWMGGIIPIFGTANYAQKFQGRVTITADESTSTAYMELSSLRSEDTAVYYCARGRAGGSWEFDYWGQGTLVTVSSGSASAPKLEEGEFSEARVEIVLTQSPSSLSASVRDRVTITCRASQSISSYLNWYQQKPGKAPKLLIYAASSLQSGVPSRFSGSGSGTDFTLTISSLQPEDFATYYCQQSYSTPFTFGPGTKVDIKRTV

SEQ ID NO: 5 - protein, 240 aa, synthetic construct
QVQLVQSGAEVKKPGASVKVSCKASGYTFTGYYMHWVRQAPGQGLEWMGWINPNSGGTNYAQEFQGRVTMTRDTSISTAYMELSRLRSDDTAVYYCLIGDYWGQGTLVTVSSGGGGSGGGGSGGGGSQSVLTQPPSASGPPGQRVTISCSGSSSNIGSNVLSWYQQVPGTAPRVLIHSNKQRPSGVPDRISASKSGTSASLTISELRSEDEAVYYCLTWDDSLDGPVFGGGTKLTVLGQP